European Patent Application EP 4 534 669 A1, published April 9, 2025. Title: Novel Modified Poly-Adenine Sequences and Uses thereof. Applicant: KAIST ITVC. Application KR. The sequence listing filed with the application follows.

SEQUENCE LISTING (28 sequences)

SEQ ID NO: 1 - DNA, 1848 bp, synthetic construct
  misc_feature 1..1848: note = luciferase-pcDNA3
  source 1..1848: mol_type = other DNA
aaatataagagccaccatggaagacgccaaaaacataaagaaaggcccggcgccattctatccgctggaagatggaaccgctggagagcaactgcataaggctatgaagagatacgccctggttcctggaacaattgcttttacagatgcacatatcgaggtggacatcacttacgctgagtacttcgaaatgtccgttcggttggcagaagctatgaaacgatatgggctgaatacaaatcacagaatcgtcgtatgcagtgaaaactctcttcaattctttatgccggtgttgggcgcgttatttatcggagttgcagttgcgcccgcgaacgacatttataatgaacgtgaattgctcaacagtatgggcatttcgcagcctaccgtggtgttcgtttccaaaaaggggttgcaaaaaattttgaacgtgcaaaaaaagctcccaatcatccaaaaaattattatcatggattctaaaacggattaccagggatttcagtcgatgtacacgttcgtcacatctcatctacctcccggttttaatgaatacgattttgtgccagagtccttcgatagggacaagacaattgcactgatcatgaactcctctggatctactggtctgcctaaaggtgtcgctctgcctcatagaactgcctgcgtgagattctcgcatgccagagatcctatttttggcaatcaaatcattccggatactgcgattttaagtgttgttccattccatcacggttttggaatgtttactacactcggatatttgatatgtggatttcgagtcgtcttaatgtatagatttgaagaagagctgtttctgaggagccttcaggattacaagattcaaagtgcgctgctggtgccaaccctattctccttcttcgccaaaagcactctgattgacaaatacgatttatctaatttacacgaaattgcttctggtggcgctcccctctctaaggaagtcggggaagcggttgccaagaggttccatctgccaggtatcaggcaaggatatgggctcactgagactacatcagctattctgattacacccgagggggatgataaaccgggcgcggtcggtaaagttgttccattttttgaagcgaaggttgtggatctggataccgggaaaacgctgggcgttaatcaaagaggcgaactgtgtgtgagaggtcctatgattatgtccggttatgtaaacaatccggaagcgaccaacgccttgattgacaaggatggatggctacattctggagacatagcttactgggacgaagacgaacacttcttcatcgttgaccgcctgaagtctctgattaagtacaaaggctatcaggtggctcccgctgaattggaatccatcttgctccaacaccccaacatcttcgacgcaggtgtcgcaggtcttcccgacgatgacgccggtgaacttcccgccgccgttgttgttttggagcacggaaagacgatgacggaaaaagagatcgtggattacgtcgccagtcaagtaacaaccgcgaaaaagttgcgcggaggagttgtgtttgtggacgaagtaccgaaaggtcttaccggaaaactcgacgcaagaaaaatcagagagatcctcataaaggccaagaagggcggaaagatcgccgtgtaattctagagggccctattctatagtgtcacctaaatgctagagctcgctgatcagcctcgactgtgccttctagttgccagccatctgttgtttgcccctcccccgtgccttccttgaccctggaaggtgccactcccactgtcctttcctaataaaatgaggaaattgcatcgcattga

SEQ ID NO: 2 - DNA, 3726 bp, synthetic construct
  source 1..3726: mol_type = other DNA
tcgcgcgtttcggtgatgacggtgaaaacctctgacacatgcagctcccggagacggtcacagcttgtctgtaagcggatgccgggagcagacaagcccgtcagggcgcgtcagcgggtgttggcgggtgtcggggctggcttaactatgcggcatcagagcagattgtactgagagtgcaccaaatgcggtgtgaaataccgcacagatgcgtaaggagaaaataccgcatcaggcgccattcgccattcaggctgcgcaactgttgggaagggcgatcggtgcgggcctcatcgctattacgccagctggcgaaagggggatgtgctgcaaggcgattaagttgggtaacgccagggttttcccagtcacgacgttgtaaaacgacggccagtgcaacgcgatgacgatggatagcgattcatcgatgagctgacccgatcgccgccgccggagggttgcgtttgagacgggcgacagatgaggctcgtttagtgaaccgtcagatcgcctggagacgccatccacgctgttttgacctccatagaagacaccgggaccgatccagcctccggactctagaggatcgaacccttttggaccctcgtacagaagctaatacgactcactataaggaaataagagagaaaagaagagtaagaagaaatataagagccaccatgggcgtgcacgagtgccccgcctggctgtggctgctgctgagcctgctgagcctgcccctgggcctgcccgtgctgggcgcccccccccggctgatctgcgacagccgggtgctggagcggtacctgctggaggccaaggaggccgagaacatcaccaccggctgcgccgagcactgcagcctgaacgagaacatcaccgtgcccgacaccaaggtgaacttctacgcctggaagcggatggaggtgggccagcaggccgtggaggtgtggcagggcctggccctgctgagcgaggccgtgctgcggggccaggccctgctggtgaacagcagccagccctgggagcccctgcagctgcacgtggacaaggccgtgagcggcctgcggagcctgaccaccctgctgcgggccctgggcgcccagaaggaggccatcagcccccccgacgccgccagcgccgcccccctgcggaccatcaccgccgacaccttccggaagctgttccgggtgtacagcaacttcctgcggggcaagctgaagctgtacaccggcgaggcctgccggaccggcgaccggtgattctagagggccctattctatagtgtcacctaaatgctagagctcgctgatcagcctcgactgtgccttctagttgccagccatctgttgtttgcccctcccccgtgccttccttgaccctggaaggtgccactcccactgtcctttcctaataaaatgaggaaattgcatcgcattgactagtgtcgacgcaaatcagttctggaccagcgagctgtgctgcgactcgtggcgtaatcatggtcatagctgtttcctgtgtgaaattgttatccgctcacaattccacacaacatacgagccggaagcataaagtgtaaagcctggggtgcctaatgagtgagctaactcacattaattgcgttgcgctcactgcccgctttccagtcgggaaacctgtcgtgccagctgcattaatgaatcggccaacgcgcggggagaggcggtttgcgtattgggcgctcttccgcttcctcgctcactgactcgctgcgctcggtcgttcggctgcggcgagcggtatcagctcactcaaaggcggtaatacggttatccacagaatcaggggataacgcaggaaagaacatgtgagcaaaaggccagcaaaaggccaggaaccgtaaaaaggccgcgttgctggcgtttttccataggctccgcccccctgacgagcatcacaaaaatcgacgctcaagtcagaggtggcgaaacccgacaggactataaagataccaggcgtttccccctggaagctccctcgtgcgctctcctgttccgaccctgtcgcttaccggatacctgtccgcctttctcccttcgggaagcgtggcgctttctcatagctcacgctgtaggtatctcagttcggtgtaggtcgttcgctccaagctgggctgtgtgcacgaaccccccgttcagcccgaccgctgcgccttatccggtaactatcgtcttgagtccaacccggtaagacacgacttatcgccactggcagcagccactggtaacaggattagcagagcgaggtatgtaggcggtgctacagagttcttgaagtggtggcctaactacggctacactagaagaacagtatttggtatctgcgctctgctgaagccagttaccttcggaaaaagagttggtagctcttgatccggcaaacaaaccaccgctggtagcggtggtttttttgtttgcaagcagcagattacgcgcagaaaaaaaggatctcaagaagatcctttgatcttttctacggggtctgacgctcagtggaacgaaaactcacgttaagggattttggtcatgagattatcaaaaaggatcttcacctagatccttttaaattaaaaatgaagttttaaatcaatctaaagtatatatgagtaaacttggtctgacagttaccaatgcttaatcagtgaggcacctatctcagcgatctgtctatttcgttcatccatagttgcctgactccccgtcgtgtagataactacgatacgggagggcttaccatctggccccagtgctgcaatgataccgcgagacccacgctcaccggctccagatttatcagcaataaaccagccagccggaagggccgagcgcagaagtggtcctgcaactttatccgcctccatccagtctattaattgttgccgggaagctagagtaagtagttcgccagttaatagtttgcgcaacgttgttgccattgctacaggcatcgtggtgtcacgctcgtcgtttggtatggcttcattcagctccggttcccaacgatcaaggcgagttacatgatcccccatgttgtgcaaaaaagcggttagctccttcggtcctccgatcgttgtcagaagtaagttggccgcagtgttatcactcatggttatggcagcactgcataattctcttactgtcatgccatccgtaagatgcttttctgtgactggtgagtactcaaccaagtcattctgagaatagtgtatgcggcgaccgagttgctcttgcccggcgtcaatacgggataataccgcgccacatagcagaactttaaaagtgctcatcattggaaaacgttcttcggggcgaaaactctcaaggatcttaccgctgttgagatccagttcgatgtaacccactcgtgcacccaactgatcttcagcatcttttactttcaccagcgtttctgggtgagcaaaaacaggaaggcaaaatgccgcaaaaaagggaataagggcgacacggaaatgttgaatactcatactctacctttttcaatattattgaagcatttatcagggttattgtctcatgagcggatacatatttgaatgtatttagaaaaataaacaaataggggttccgcgcacatttccccgaaaagtgccacctgacgtctaagaaaccattattatcatgacattaacctataaaaataggcgtatcacgaggccctttcgtc

SEQ ID NO: 3 - DNA, 2969 bp, synthetic construct
  misc_feature 1..2969: note = GFP-pUC
  source 1..2969: mol_type = other DNA
ctagtgtcgacgcaaatcagttctggaccagcgagctgtgctgcgactcgtggcgtaatcatggtcatagctgtttcctgtgtgaaattgttatccgctcacaattccacacaacatacgagccggaagcataaagtgtaaagcctggggtgcctaatgagtgagctaactcacattaattgcgttgcgctcactgcccgctttccagtcgggaaacctgtcgtgccagctgcattaatgaatcggccaacgcgcggggagaggcggtttgcgtattgggcgctcttccgcttcctcgctcactgactcgctgcgctcggtcgttcggctgcggcgagcggtatcagctcactcaaaggcggtaatacggttatccacagaatcaggggataacgcaggaaagaacatgtgagcaaaaggccagcaaaaggccaggaaccgtaaaaaggccgcgttgctggcgtttttccataggctccgcccccctgacgagcatcacaaaaatcgacgctcaagtcagaggtggcgaaacccgacaggactataaagataccaggcgtttccccctggaagctccctcgtgcgctctcctgttccgaccctgtcgcttaccggatacctgtccgcctttctcccttcgggaagcgtggcgctttctcatagctcacgctgtaggtatctcagttcggtgtaggtcgttcgctccaagctgggctgtgtgcacgaaccccccgttcagcccgaccgctgcgccttatccggtaactatcgtcttgagtccaacccggtaagacacgacttatcgccactggcagcagccactggtaacaggattagcagagcgaggtatgtaggcggtgctacagagttcttgaagtggtggcctaactacggctacactagaagaacagtatttggtatctgcgctctgctgaagccagttaccttcggaaaaagagttggtagctcttgatccggcaaacaaaccaccgctggtagcggtggtttttttgtttgcaagcagcagattacgcgcagaaaaaaaggatctcaagaagatcctttgatcttttctacggggtctgacgctcagtggaacgaaaactcacgttaagggattttggtcatgagattatcaaaaaggatcttcacctagatccttttaaattaaaaatgaagttttaaatcaatctaaagtatatatgagtaaacttggtctgacagttaccaatgcttaatcagtgaggcacctatctcagcgatctgtctatttcgttcatccatagttgcctgactccccgtcgtgtagataactacgatacgggagggcttaccatctggccccagtgctgcaatgataccgcgagacccacgctcaccggctccagatttatcagcaataaaccagccagccggaagggccgagcgcagaagtggtcctgcaactttatccgcctccatccagtctattaattgttgccgggaagctagagtaagtagttcgccagttaatagtttgcgcaacgttgttgccattgctacaggcatcgtggtgtcacgctcgtcgtttggtatggcttcattcagctccggttcccaacgatcaaggcgagttacatgatcccccatgttgtgcaaaaaagcggttagctccttcggtcctccgatcgttgtcagaagtaagttggccgcagtgttatcactcatggttatggcagcactgcataattctcttactgtcatgccatccgtaagatgcttttctgtgactggtgagtactcaaccaagtcattctgagaatagtgtatgcggcgaccgagttgctcttgcccggcgtcaatacgggataataccgcgccacatagcagaactttaaaagtgctcatcattggaaaacgttcttcggggcgaaaactctcaaggatcttaccgctgttgagatccagttcgatgtaacccactcgtgcacccaactgatcttcagcatcttttactttcaccagcgtttctgggtgagcaaaaacaggaaggcaaaatgccgcaaaaaagggaataagggcgacacggaaatgttgaatactcatactctacctttttcaatattattgaagcatttatcagggttattgtctcatgagcggatacatatttgaatgtatttagaaaaataaacaaataggggttccgcgcacatttccccgaaaagtgccacctgacgtctaagaaaccattattatcatgacattaacctataaaaataggcgtatcacgaggccctttcgtctcgcgcgtttcggtgatgacggtgaaaacctctgacacatgcagctcccggagacggtcacagcttgtctgtaagcggatgccgggagcagacaagcccgtcagggcgcgtcagcgggtgttggcgggtgtcggggctggcttaactatgcggcatcagagcagattgtactgagagtgcaccaaatgcggtgtgaaataccgcacagatgcgtaaggagaaaataccgcatcaggcgccattcgccattcaggctgcgcaactgttgggaagggcgatcggtgcgggcctcatcgctattacgccagctggcgaaagggggatgtgctgcaaggcgattaagttgggtaacgccagggttttcccagtcacgacgttgtaaaacgacggccagtgcaacgcgatgacgatggatagcgattcatcgatgagctgacccgatcgccgccgccggagggttgcgtttgagacgggcgacagatgaggctcgtttagtgaaccgtcagatcgcctggagacgccatccacgctgttttgacctccatagaagacaccgggaccgatccagcctccggactctagaggatcgaacccttttggaccctcgtacagaagctaatacgactcactatagggaaataagagagaaaagaagagtaagaagaaatataagagccaccatgg

SEQ ID NO: 4 - DNA, 27 bp, synthetic construct
  misc_feature 1..27: note = Forward primer-luciferase-pcDNA3
  source 1..27: mol_type = other DNA
aaatataagagccaccatggaagacgc

SEQ ID NO: 5 - DNA, 134 bp, synthetic construct
  misc_feature 1..134: note = Reverse primer- luciferase-pcDNA3 <A(10)G(1)-76>
  source 1..134: mol_type = other DNA
tgatttgcgtcgacactagtggtctctttttttttttcttttttttttcttttttttttcttttttttttcttttttttttcttttttttttcttttttttttcaatgcgatgcaatttcctcattttattagg

SEQ ID NO: 6 - DNA, 200 bp, synthetic construct
  misc_feature 1..200: note = Reverse primer- luciferase-pcDNA3 <A(10)G(1)-142>
  source 1..200: mol_type = other DNA
tgatttgcgtcgacactagtggtctctttttttttttcttttttttttcttttttttttcttttttttttcttttttttttcttttttttttcttttttttttcttttttttttcttttttttttcttttttttttcttttttttttcttttttttttcttttttttttcaatgcgatgcaatttcctcattttattagg

SEQ ID NO: 7 - DNA, 245 bp, synthetic construct
  misc_feature 1..245: note = Reverse primer- luciferase-pcDNA3 <A(10)G(1)-186>
  source 1..245: mol_type = other DNA
tgatttgcgtcgacactagtggtctctttttttttttcttttttttttcttttttttttcttttttttttcttttttttttcttttttttttcttttttttttcttttttttttcttttttttttcttttttttttcttttttttttcttttttttttcttttttttttcttttttttttcttttttttttcttttttttttctttttttttttcaatgcgatgcaatttcctcattttattagg

SEQ ID NO: 8 - DNA, 200 bp, synthetic construct
  misc_feature 1..200: note = Reverse primer- luciferase-pcDNA3 <A(10)C(1)-142>
  source 1..200: mol_type = other DNA
tgatttgcgtcgacactagtggtctctttttttttttgttttttttttgttttttttttgttttttttttgttttttttttgttttttttttgttttttttttgttttttttttgttttttttttgttttttttttgttttttttttgttttttttttgttttttttttcaatgcgatgcaatttcctcattttattagg

SEQ ID NO: 9 - DNA, 200 bp, synthetic construct
  misc_feature 1..200: note = Reverse primer- luciferase-pcDNA3 <A(15)G(1)-142>
  source 1..200: mol_type = other DNA
tgatttgcgtcgacactagtggtctctttttttttttttttctttttttttttttttctttttttttttttttctttttttttttttttctttttttttttttttctttttttttttttttctttttttttttttttctttttttttttttttctttttttttttttttcaatgcgatgcaatttcctcattttattagg

SEQ ID NO: 10 - DNA, 200 bp, synthetic construct
  misc_feature 1..200: note = Reverse primer- luciferase-pcDNA3 <A(15)G(2)-142>
  source 1..200: mol_type = other DNA
tgatttgcgtcgacactagtggtctctttttttcctttttttttttttttcctttttttttttttttcctttttttttttttttcctttttttttttttttcctttttttttttttttcctttttttttttttttcctttttttttttttttcctttttttttttttttcaatgcgatgcaatttcctcattttattagg

SEQ ID NO: 11 - DNA, 200 bp, synthetic construct
  misc_feature 1..200: note = Reverse primer- luciferase-pcDNA3 <A(20)G(1)-142>
  source 1..200: mol_type = other DNA
tgatttgcgtcgacactagtggtctctttttttttttttttttcttttttttttttttttttttcttttttttttttttttttttcttttttttttttttttttttcttttttttttttttttttttcttttttttttttttttttttcttttttttttttttttttttcaatgcgatgcaatttcctcattttattagg

SEQ ID NO: 12 - DNA, 200 bp, synthetic construct
  misc_feature 1..200: note = Reverse primer- luciferase-pcDNA3 <A(30)G(1)-142>
  source 1..200: mol_type = other DNA
tgatttgcgtcgacactagtggtctctttttttttttttttttttcttttttttttttttttttttttttttttttcttttttttttttttttttttttttttttttcttttttttttttttttttttttttttttttcttttttttttttttttttttttttttttttcaatgcgatgcaatttcctcattttattagg

SEQ ID NO: 13 - DNA, 200 bp, synthetic construct
  misc_feature 1..200: note = Reverse primer- luciferase-pcDNA3 <A(30)G(2)-142>
  source 1..200: mol_type = other DNA
tgatttgcgtcgacactagtggtctctttttttttttttttccttttttttttttttttttttttttttttttccttttttttttttttttttttttttttttttccttttttttttttttttttttttttttttttccttttttttttttttttttttttttttttttcaatgcgatgcaatttcctcattttattagg

SEQ ID NO: 14 - DNA, 200 bp, synthetic construct
  misc_feature 1..200: note = Reverse primer- luciferase-pcDNA3 <A(5)G(1)-142>
  source 1..200: mol_type = other DNA
tgatttgcgtcgacactagtggtctctttttctttttctttttctttttctttttctttttctttttctttttctttttctttttctttttctttttctttttctttttctttttctttttctttttctttttctttttctttttctttttctttttctttttctttttcaatgcgatgcaatttcctcattttattagg

SEQ ID NO: 15 - DNA, 200 bp, synthetic construct
  misc_feature 1..200: note = Reverse primer- luciferase-pcDNA3 <A(3)G(1)-142>
  source 1..200: mol_type = other DNA
tgatttgcgtcgacactagtggtctctttctttctttctttctttctttctttctttctttctttctttctttctttctttctttctttctttctttctttctttctttctttctttctttctttctttctttctttctttctttctttctttctttctttctttctttcaatgcgatgcaatttcctcattttattagg

SEQ ID NO: 16 - DNA, 200 bp, synthetic construct
  misc_feature 1..200: note = Reverse primer- luciferase-pcDNA3 <A(10)G(2)-142>
  source 1..200: mol_type = other DNA
tgatttgcgtcgacactagtggtctctttttttttttccttttttttttccttttttttttccttttttttttccttttttttttccttttttttttccttttttttttccttttttttttccttttttttttccttttttttttccttttttttttccttttttttttcaatgcgatgcaatttcctcattttattagg

SEQ ID NO: 17 - DNA, 200 bp, synthetic construct
  misc_feature 1..200: note = Reverse primer- luciferase-pcDNA3 <A(10)G(3)-142>
  source 1..200: mol_type = other DNA
tgatttgcgtcgacactagtggtctctccttttttttttcccttttttttttcccttttttttttcccttttttttttcccttttttttttcccttttttttttcccttttttttttcccttttttttttcccttttttttttcccttttttttttcccttttttttttcaatgcgatgcaatttcctcattttattagg

SEQ ID NO: 18 - DNA, 167 bp, synthetic construct
  source 1..167: mol_type = other DNA
tgatttgcgtcgacactagtggtctctttttttttttcttttttttttcttttttttttcttttttttttcttttttttttcttttttttttcttttttttttcttttttttttcttttttttttcttttttttttcaatgcgatgcaatttcctcattttattagg

SEQ ID NO: 19 - DNA, 178 bp, synthetic construct
  source 1..178: mol_type = other DNA
tgatttgcgtcgacactagtggtctctttttttttttcttttttttttcttttttttttcttttttttttcttttttttttcttttttttttcttttttttttcttttttttttcttttttttttcttttttttttcttttttttttcaatgcgatgcaatttcctcattttattagg

SEQ ID NO: 20 - DNA, 181 bp, synthetic construct
  source 1..181: mol_type = other DNA
tgatttgcgtcgacactagtggtctctttttttttttcttttttttttcttttttttttcttttttttttcttttttttttcttttttttttcttttttttttcttttttttttcttttttttttcttttttttttcttttttttttcttcaatgcgatgcaatttcctcattttattagg

SEQ ID NO: 21 - DNA, 189 bp, synthetic construct
  source 1..189: mol_type = other DNA
tgatttgcgtcgacactagtggtctctttttttttttcttttttttttcttttttttttcttttttttttcttttttttttcttttttttttcttttttttttcttttttttttcttttttttttcttttttttttcttttttttttcttttttttttcaatgcgatgcaatttcctcattttattagg

SEQ ID NO: 22 - DNA, 200 bp, synthetic construct
  source 1..200: mol_type = other DNA
tgatttgcgtcgacactagtggtctcttttttttcttttttttcttttttttcttttttttcttttttttcttttttttcttttttttcttttttttcttttttttcttttttttcttttttttcttttttttcttttttttcttttttttcttttttttcttttttttcaatgcgatgcaatttcctcattttattagg

SEQ ID NO: 23 - DNA, 200 bp, synthetic construct
  source 1..200: mol_type = other DNA
tgatttgcgtcgacactagtggtctctttttttttttattttttttttattttttttttattttttttttattttttttttattttttttttattttttttttattttttttttattttttttttattttttttttattttttttttattttttttttattttttttttcaatgcgatgcaatttcctcattttattagg

SEQ ID NO: 24 - DNA, 200 bp, synthetic construct
  source 1..200: mol_type = other DNA
tgatttgcgtcgacactagtggtctctttttttttttcttttttttttgttttttttttcttttttttttgttttttttttcttttttttttgttttttttttcttttttttttgttttttttttcttttttttttgttttttttttcttttttttttgttttttttttcaatgcgatgcaatttcctcattttattagg

SEQ ID NO: 25 - DNA, 200 bp, synthetic construct
  source 1..200: mol_type = other DNA
tgatttgcgtcgacactagtggtctctttttttttttcttttttttttattttttttttcttttttttttattttttttttcttttttttttattttttttttcttttttttttattttttttttcttttttttttattttttttttcttttttttttattttttttttcaatgcgatgcaatttcctcattttattagg

SEQ ID NO: 26 - DNA, 167 bp, synthetic construct
  source 1..167: mol_type = other DNA
tgatttgcgtcgacactagtggtctcttttttttttttttttttttttttttttttttttttttttttttttttttttttttttttttttttttttagtcatatgcttttttttttttttttttttttttttttttcaatgcgatgcaatttcctcattttattagg

SEQ ID NO: 27 - DNA, 24 bp, synthetic construct
  misc_feature 1..24: note = Forward primer-GFP-pUC
  source 1..24: mol_type = other DNA
ctagtgtcgacgcaaatcagttct

SEQ ID NO: 28 - DNA, 28 bp, synthetic construct
  misc_feature 1..28: note = Reverse primer-GFP-pUC
  source 1..28: mol_type = other DNA
ccatggtggctcttatatttcttcttac